European Patent Application EP 4 454 663 A1, published October 30, 2024. Title: DIAGNOSTIC METHODS, THERAPEUTIC AND PROPHYLACTIC AGENTS FOR HEART FAILURE, MYOCARDIAL INFARCTION AND CARDIAC FIBROSIS. Applicant: 国立大学法人　東京大学. Application JP. The sequence listing filed with the application follows.

SEQUENCE LISTING (14 sequences)

SEQ ID NO: 1 - DNA, 20 bp, synthetic construct
  source 1..20: mol_type = other DNA
tcctggcagagaggaggaag

SEQ ID NO: 2 - DNA, 20 bp, synthetic construct
  source 1..20: mol_type = other DNA
tgcaggtcgaacttctcagc

SEQ ID NO: 3 - DNA, 20 bp, synthetic construct
  source 1..20: mol_type = other DNA
caactgggacgacatggaga

SEQ ID NO: 4 - DNA, 20 bp, synthetic construct
  source 1..20: mol_type = other DNA
gcatacagggacagcacagc

SEQ ID NO: 5 - DNA, 21 bp, synthetic construct
  source 1..21: mol_type = other DNA
aagtgggaagaggcagactga

SEQ ID NO: 6 - DNA, 19 bp, synthetic construct
  source 1..19: mol_type = other DNA
gtcaatggccagcaccttc

SEQ ID NO: 7 - DNA, 19 bp, synthetic construct
  source 1..19: mol_type = other DNA
cttagagggacaagtggcg

SEQ ID NO: 8 - DNA, 20 bp, synthetic construct
  source 1..20: mol_type = other DNA
acgctgagccagtcagtgta

SEQ ID NO: 9 - DNA, 20 bp, synthetic construct
  source 1..20: mol_type = other DNA
tgaccagtccgcggtacaag

SEQ ID NO: 10 - DNA, 20 bp, synthetic construct
  source 1..20: mol_type = other DNA
ttggagctggagaccacgtg

SEQ ID NO: 11 - DNA, 19 bp, synthetic construct
  source 1..19: mol_type = other DNA
ctcccgtggcttctagtgc

SEQ ID NO: 12 - DNA, 22 bp, synthetic construct
  source 1..22: mol_type = other DNA
gccttagtttggacaggatctg

SEQ ID NO: 13 - protein, 12 aa, Homo sapiens
CVKSRKRRKGKA

SEQ ID NO: 14 - protein, 9 aa, Homo sapiens
CPLGETRDA